European Patent Application EP 4 137 519 A1, published February 22, 2023. Title: COMBINATION OF IFN-GAMMA WITH ANTI-ERBB ANTIBODY FOR THE TREATMENT OF CANCERS. Applicant: The Trustees of the University of Pennsylvania. The sequence listing filed with the application follows.

SEQUENCE LISTING (9 sequences)

SEQ ID NO: 1 - protein, 324 aa, synthetic construct
  REGION 1..324: note = 4D5scFvZZ
MADIQMTQSPSSLSASVGDRVTITCRASQDVNTAVAWYQQKPGKAPKLLIYSASFLYSGVPSRFSGSRSGTDFTLTISSLQPEDFATYYCQQHYTTPPTFGQGTKVELKRATPSHNSHQVPSAGGPTANSGEVKLVESGGGLVQPGGSLRLSCATSGFNIKDTYIHWVRQAPGKGLEWVARIYPTNGYTRYADSVKGRFTISADTSKNTAYLQMNSLRAEDTAVYYCSRWGGDGFYAMDYWGQGTTVTVSSGGGGSVDVDNKFNKEQQNAFYEILHLPNLNEEQRNAFIQSLKDDPSQSANLLAEAKKLNDAQAPKLEHHHHHH

SEQ ID NO: 2 - protein, 464 aa, synthetic construct
  REGION 1..464: note = 4D5scFvZZ-IFN-gamma
MADIQMTQSPSSLSASVGDRVTITCRASQDVNTAVAWYQQKPGKAPKLLIYSASFLYSGVPSRFSGSRSGTDFTLTISSLQPEDFATYYCQQHYTTPPTFGQGTKVELKRATPSHNSHQVPSAGGPTANSGEVKLVESGGGLVQPGGSLRLSCATSGFNIKDTYIHWVRQAPGKGLEWVARIYPTNGYTRYADSVKGRFTISADTSKNTAYLQMNSLRAEDTAVYYCSRWGGDGFYAMDYWGQGTTVTVSSGGGGSVDVDNKFNKEQQNAFYEILHLPNLNEEQRNAFIQSLKDDPSQSANLLAEAKKLNDAQAPKLEGGGGSQDPYVKEAENLKKYFNAGHSDVADNGTLFLGILKNWKEESDRKIMQSQIVSFYFKLFKNFKDDQSIQKSVETIKEDMNVKFFNSNKKKRDDFEKLTNYSVTDLNVQRKAIHELIQVMAELSPAAKTGKRKRSQLEHHHHHH

SEQ ID NO: 3 - protein, 259 aa, synthetic construct
  REGION 1..259: note = 4D5scFv
MADIQMTQSPSSLSASVGDRVTITCRASQDVNTAVAWYQQKPGKAPKLLIYSASFLYSGVPSRFSGSRSGTDFTLTISSLQPEDFATYYCQQHYTTPPTFGQGTKVELKRATPSHNSHQVPSAGGPTANSGEVKLVESGGGLVQPGGSLRLSCATSGFNIKDTYIHWVRQAPGKGLEWVARIYPTNGYTRYADSVKGRFTISADTSKNTAYLQMNSLRAEDTAVYYCSRWGGDGFYAMDYWGQGTTVTVSSLEHHHHHH

SEQ ID NO: 4 - protein, 61 aa, synthetic construct
  REGION 1..61: note = ZZ
SVDVDNKFNKEQQNAFYEILHLPNLNEEQRNAFIQSLKDDPSQSANLLAEAKKLNDAQAPK

SEQ ID NO: 5 - protein, 133 aa, synthetic construct
  REGION 1..133: note = IFN-gamma
QDPYVKEAENLKKYFNAGHSDVADNGTLFLGILKNWKEESDRKIMQSQIVSFYFKLFKNFKDDQSIQKSVETIKEDMNVKFFNSNKKKRDDFEKLTNYSVTDLNVQRKAIHELIQVMAELSPAAKTGKRKRSQ

SEQ ID NO: 6 - protein, 5 aa, synthetic construct
  REGION 1..5: note = Glycine-serine oligopeptide linker
GGGGS

SEQ ID NO: 7 - protein, 6 aa, synthetic construct
  REGION 1..6: note = Glycine-serine oligopeptide linker
GGGGGS

SEQ ID NO: 8 - DNA, 28 bp, synthetic construct
  misc_feature 1..28: note = snail 6SA insert forward primer
  source 1..28: mol_type = other DNA
aaagaagcttatgccgcgctctttcctc

SEQ ID NO: 9 - DNA, 32 bp, synthetic construct
  misc_feature 1..32: note = snail 6SA insert reverse primer
  source 1..32: mol_type = other DNA
aaagtctagatcagcggggacatcctgagcag